European Patent Specification EP 4 055 190 B1, published July 3, 2024. Title: Diagnosis of mood disorders using blood RNA editing biomarkers. Applicant: ALCEDIAG. The sequence listing filed with the application follows.

SEQUENCE LISTING (36 sequences)

SEQ ID NO: 1 - RNA, 23 nt, Homo sapiens
atacgggcaagctcttaactatt

SEQ ID NO: 2 - RNA, 20 nt, Homo sapiens
aacctccacctcctgttttc

SEQ ID NO: 3 - RNA, 23 nt, Homo sapiens
aaaatacgggcaagctcttaact

SEQ ID NO: 4 - RNA, 20 nt, Homo sapiens
ctgcacttaggctcacagga

SEQ ID NO: 5 - RNA, 21 nt, Homo sapiens
atgcaagttgtggacatggag

SEQ ID NO: 6 - RNA, 21 nt, Homo sapiens
ttctgaaaacaatgggcacca

SEQ ID NO: 7 - RNA, 19 nt, Homo sapiens
tgtgcaaagggctccatac

SEQ ID NO: 8 - RNA, 21 nt, Homo sapiens
ccttgcaagtgtccagtaaac

SEQ ID NO: 9 - RNA, 20 nt, Homo sapiens
ctagggtgaggtggtgcaat

SEQ ID NO: 10 - RNA, 20 nt, Homo sapiens
caaggccaggagttcaagac

SEQ ID NO: 11 - RNA, 22 nt, Homo sapiens
tttaaaagcttctccagtcagc

SEQ ID NO: 12 - RNA, 27 nt, Homo sapiens
caagactgagcatacattatattcacc

SEQ ID NO: 13 - RNA, 22 nt, Homo sapiens
tttaaaagcttctccagtcagc

SEQ ID NO: 14 - RNA, 20 nt, Homo sapiens
tcctgagtagctgggaccat

SEQ ID NO: 15 - RNA, 20 nt, Homo sapiens
cagcacattctgttgccttc

SEQ ID NO: 16 - RNA, 20 nt, Homo sapiens
gtgactttgcccctcatttg

SEQ ID NO: 17 - RNA, 23 nt, Homo sapiens
ggccactctgtactatgcaaatc

SEQ ID NO: 18 - RNA, 21 nt, Homo sapiens
tgaatttcagatggacagcaa

SEQ ID NO: 19 - RNA, 21 nt, Homo sapiens
aagcccatcctcgaactacag

SEQ ID NO: 20 - RNA, 20 nt, Homo sapiens
ttgctctgtcacctggactg

SEQ ID NO: 21 - RNA, 20 nt, Homo sapiens
gaaccaggctaggtgcaatg

SEQ ID NO: 22 - RNA, 20 nt, Homo sapiens
ccatgccctggtaatttttg

SEQ ID NO: 23 - RNA, 23 nt, Homo sapiens
tctgatggaatcccaaactgaga

SEQ ID NO: 24 - RNA, 24 nt, Homo sapiens
tcagagatattttgtccgaagcca

SEQ ID NO: 25 - RNA, 20 nt, Homo sapiens
cccacagtttcagaggtggt

SEQ ID NO: 26 - RNA, 18 nt, Homo sapiens
ggctcacccctgtaatcc

SEQ ID NO: 27 - RNA, 20 nt, Homo sapiens
gggatgtaaacgctgaatgg

SEQ ID NO: 28 - RNA, 20 nt, Homo sapiens
atgtgccaccatgactgact

SEQ ID NO: 29 - RNA, 20 nt, Homo sapiens
cccttccggcaagaatccag

SEQ ID NO: 30 - RNA, 20 nt, Homo sapiens
acccaagctgcataaaaggc

SEQ ID NO: 31 - RNA, 24 nt, Homo sapiens
gcaaccttagatctcaatggctaa

SEQ ID NO: 32 - RNA, 21 nt, Homo sapiens
agcagagtcacagtctacagc

SEQ ID NO: 33 - RNA, 20 nt, Homo sapiens
ccggggctcatttataggat

SEQ ID NO: 34 - RNA, 20 nt, Homo sapiens
tgctagataccgccacattg

SEQ ID NO: 35 - RNA, 20 nt, Homo sapiens
taaggacggagttcgagacc

SEQ ID NO: 36 - RNA, 21 nt, Homo sapiens
tgagagagttttgctctgtgg